European Patent Application EP 4 600 373 A1, published August 13, 2025. Title: DATA COLLECTION METHOD AND KIT FOR DETERMINING LIKELIHOOD OF DEVELOPING ALZHEIMER'S DISEASE. Applicant: KOBAYASHI Nobuyuki. Application EP 23874953.5, filed October 6, 2023. The sequence listing filed with the application follows.

SEQUENCE LISTING (9 sequences)

SEQ ID NO: 1 - DNA, 191 bp, Homo sapiens
  source 1..191: mol_type = genomic DNA
gattatgggataggagaagtgcccgtggagcccctggatgtccccttaccctccacgatcaggccagcttcccccgtggccgggtctccaaagcagccggtgcgtggctactaccgtggcgctgtcggtggcacgtttgaccgcctgcacaacgcccacaaggtgttgctcagtgtcgcgtgcatcctggc

SEQ ID NO: 2 - DNA, 21 bp, synthetic construct
  source 1..21: mol_type = other DNA
gattatgggataggagaagtg

SEQ ID NO: 3 - DNA, 24 bp, synthetic construct
  source 1..24: mol_type = other DNA
aactactcctaaaccaaaatacac

SEQ ID NO: 4 - DNA, 33 bp, synthetic construct
  source 1..33: mol_type = other DNA
tcgtggagtttttggatgtttttttatttttta

SEQ ID NO: 5 - DNA, 33 bp, synthetic construct
  source 1..33: mol_type = other DNA
ttgtggagtttttggatgtttttttatttttta

SEQ ID NO: 6 - DNA, 23 bp, synthetic construct
  source 1..23: mol_type = other DNA
gattatgggataggagaagtgtt

SEQ ID NO: 7 - DNA, 22 bp, synthetic construct
  source 1..22: mol_type = other DNA
cctaatccaaaatccctcttac

SEQ ID NO: 8 - DNA, 18 bp, synthetic construct
  source 1..18: mol_type = other DNA
accacaaactactcctaa

SEQ ID NO: 9 - DNA, 21 bp, synthetic construct
  source 1..21: mol_type = other DNA
caccacaaactactcctaaac